European Patent Specification EP 3 646 883 B1, published October 18, 2023. Title: A NOVEL TUMOR VACCINE AND USES THEREOF. Applicant: Sichuan University. The sequence listing filed with the application follows.

SEQUENCE LISTING (11 sequences)

SEQ ID NO: 1 - DNA, 1978 bp, Artificial Sequence
  nucleotide sequence of pMVA
gactcttcgcgatgtacgggccagatatacgccttctactgggcggttttatggacagcaagcgaaccggaattgccagctggggcgccctctggtaaggttgggaagccctgcaaagtaaactggatggctttctcgccgccaaggatctgatggcgcaggggatcaagctctgatcaagagacaggatgaggatcgtttcgcatgattgaacaagatggattgcacgcaggttctccggccgcttgggtggagaggctattcggctatgactgggcacaacagacaatcggctgctctgatgccgccgtgttccggctgtcagcgcaggggcgcccggttctttttgtcaagaccgacctgtccggtgccctgaatgaactgcaagacgaggcagcgcggctatcgtggctggccacgacgggcgttccttgcgcagctgtgctcgacgttgtcactgaagcgggaagggactggctgctattgggcgaagtgccggggcaggatctcctgtcatctcaccttgctcctgccgagaaagtatccatcatggctgatgcaatgcggcggctgcatacgcttgatccggctacctgcccattcgaccaccaagcgaaacatcgcatcgagcgagcacgtactcggatggaagccggtcttgtcgatcaggatgatctggacgaagagcatcaggggctcgcgccagccgaactgttcgccaggctcaaggcgagcatgcccgacggcgaggatctcgtcgtgacccatggcgatgcctgcttgccgaatatcatggtggaaaatggccgcttttctggattcatcgactgtggccggctgggtgtggcggaccgctatcaggacatagcgttggctacccgtgatattgctgaagagcttggcggcgaatgggctgaccgcttcctcgtgctttacggtatcgccgctcccgattcgcagcgcatcgccttctatcgccttcttgacgagttcttctgaattattaacgcttacaatttcctgatgcggtattttctccttacgcatctgtgcggtatttcacaccgcatacaggtggcacttttcggggaaatgtgcgcggaacccctatttgtttatttttctaaatacattcaaatatgtatccgctcatgagacaataaccctgataaatgcttcaataatagcacgtgctaaaacttcatttttaatttaaaaggatctaggtgaagatcctttttgataatctcatgaccaaaatcccttaacgtgagttttcgttccactgagcgtcagaccccgtagaaaagatcaaaggatcttcttgagatcctttttttctgcgcgtaatctgctgcttgcaaacaaaaaaaccaccgctaccagcggtggtttgtttgccggatcaagagctaccaactctttttccgaaggtaactggcttcagcagagcgcagataccaaatactgtccttctagtgtagccgtagttaggccaccacttcaagaactctgtagcaccgcctacatacctcgctctgctaatcctgttaccagtggctgctgccagtggcgataagtcgtgtcttaccgggttggactcaagacgatagttaccggataaggcgcagcggtcgggctgaacggggggttcgtgcacacagcccagcttggagcgaacgacctacaccgaactgagatacctacagcgtgagctatgagaaagcgccacgcttcccgaagggagaaaggcggacaggtatccggtaagcggcagggtcggaacaggagagcgcacgagggagcttccagggggaaacgcctggtatctttatagtcctgtcgggtttcgccacctctgacttgagcgtcgatttttgtgatgctcgtcaggggggcggagcctatggaaaaacgccagcaacgcggcctttttacggttcctgggcttttgctggccttttgctcacatgttctt

SEQ ID NO: 2 - DNA, 1977 bp, Artificial Sequence
  nucleotide sequence of pMVA
gctgcttcgcgatgtacgggccagatatacgccttctactgggcggttttatggacagcaagcgaaccggaattgccagctggggcgccctctggtaaggttgggaagccctgcaaagtaaactggatggctttcttgccgccaaggatctgatggcgcaggggatcaagctctgatcaagagacaggatgaggatcgtttcgcatgattgaacaagatggattgcacgcaggttctccggccgcttgggtggagaggctattcggctatgactgggcacaacagacaatcggctgctctgatgccgccgtgttccggctgtcagcgcaggggcgcccggttctttttgtcaagaccgacctgtccggtgccctgaatgaactgcaagacgaggcagcgcggctatcgtggctggccacgacgggcgttccttgcgcagctgtgctcgacgttgtcactgaagcgggaagggactggctgctattgggcgaagtgccggggcaggatctcctgtcatctcaccttgctcctgccgagaaagtatccatcatggctgatgcaatgcggcggctgcatacgcttgatccggctacctgcccattcgaccaccaagcgaaacatcgcatcgagcgagcacgtactcggatggaagccggtcttgtcgatcaggatgatctggacgaagagcatcaggggctcgcgccagccgaactgttcgccaggctcaaggcgagcatgcccgacggcgaggatctcgtcgtgacccatggcgatgcctgcttgccgaatatcatggtggaaaatggccgcttttctggattcatcgactgtggccggctgggtgtggcggaccgctatcaggacatagcgttggctacccgtgatattgctgaagagcttggcggcgaatgggctgaccgcttcctcgtgctttacggtatcgccgctcccgattcgcagcgcatcgccttctatcgccttcttgacgagttcttctgaattattaacgcttacaatttcctgatgcggtattttctccttacgcatctgtgcggtatttcacaccgcatcaggtggcacttttcggggaaatgtgcgcggaacccctatttgtttatttttctaaatacattcaaatatgtatccgctcatgagacaataaccctgataaatgcttcaataatagcacgtgctaaaacttcatttttaatttaaaaggatctaggtgaagatcctttttgataatctcatgaccaaaatcccttaacgtgagttttcgttccactgagcgtcagaccccgtagaaaagatcaaaggatcttcttgagatcctttttttctgcgcgtaatctgctgcttgcaaacaaaaaaaccaccgctaccagcggtggtttgtttgccggatcaagagctaccaactctttttccgaaggtaactggcttcagcagagcgcagataccaaatactgttcttctagtgtagccgtagttaggccaccacttcaagaactctgtagcaccgcctacatacctcgctctgctaatcctgttaccagtggctgctgccagtggcgataagtcgtgtcttaccgggttggactcaagacgatagttaccggataaggcgcagcggtcgggctgaacggggggttcgtgcacacagcccagcttggagcgaacgacctacaccgaactgagatacctacagcgtgagctatgagaaagcgccacgcttcccgaagggagaaaggcggacaggtatccggtaagcggcagggtcggaacaggagagcgcacgagggagcttccagggggaaacgcctggtatctttatagtcctgtcgggtttcgccacctctgacttgagcgtcgatttttgtgatgctcgtcaggggggcggagcctatggaaaaacgccagcaacgcggcctttttacggttcctggccttttgctggccttttgctcacatgttctt

SEQ ID NO: 3 - DNA, 120 bp, Artificial Sequence
  nucleotide sequence of pMVA
cccattattcctagaaccaggcgacctgcgactccttgacgttgacaatcgagtagtactcccgattgaagcccccattcgtataataattacatcacaagacgtcttgcactcatgagc

SEQ ID NO: 4 - DNA, 600 bp, Artificial Sequence
  nucleotide sequence of pMVA
ctgaactatcctgcccgccatcatcctagtcctcatcgccctcccatccctacgcatcctttacataacagacgaggtcaacgatccctcccttaccatcaaatcaattggccaccaatggtactgaacctacgagtacaccgactacggcggactaatcttcaactcctacatacttcccccattattcctagaaccaggcgacctgcgactccttgacgttgacaatcgagtagtactcccgattgaagcccccattcgtataataattacatcacaagacgtcttgcactcatgagctgtccccacattaggcttaaaaacagatgcaattcccggacgtctaaaccaaaccactttcaccgctacacgaccgggggtatactacggtcaatgctctgaaatctgtggagcaaaccacagtttcatgcccatcgtcctagaattaattcccctaaaaatctttgaaatagggcccgtatttaccctatagcaccccctctaccccctctagagcccactgtaaagctaacttagcattaaccttttaagttaaagattaagagaaccaacacctctttacagtgaaatgccccaact

SEQ ID NO: 5 - DNA, 2000 bp, Artificial Sequence
  nucleotide sequence of pMVA
tacgttgtagctcacttccactatgtcctatcaataggagctgtatttgccatcataggaggcttcattcactgatttcccctattctcaggctacaccctagaccaaacctacgccaaaatccatttcactatcatattcatcggcgtaaatctaactttcttcccacaacactttctcggcctatccggaatgccccgacgttactcggactaccccgatgcatacaccacatgaaacatcctatcatctgtaggctcattcatttctctaacagcagtaatattaataattttcatgatttgagaagccttcgcttcgaagcgaaaagtcctaatagtagaagaaccctccataaacctggagtgactatatggatgccccccaccctaccacacattcgaagaacccgtatacataaaatctagacaaaaaaggaaggaatcgaaccccccaaagctggtttcaagccaaccccatggcctccatgactttttcaaaaaggtattagaaaaaccatttcataactttgtcaaagttaaattataggctaaatcctatatatcttaatggcacatgcagcgcaagtaggtctacaagacgctacttcccctatcatagaagagcttatcacctttcatgatcacgccctcataatcattttccttatctgcttcctagtcctgtatgcccttttcctaacactcacaacaaaactaactaatactaacatctcagacgctcaggaaatagaaaccgtctgaactatcctgcccgccatcatcctagtcctcatcgccctcccatccctacgcatcctttacataacagacgaggtcaacgatccctcccttaccatcaaatcaattggccaccaatggtactgaacctacgagtacaccgactacggcggactaatcttcaactcctacatacttcccccattattcctagaaccaggcgacctgcgactccttgacgttgacaatcgagtagtactcccgattgaagcccccattcgtataataattacatcacaagacgtcttgcactcatgagctgtccccacattaggcttaaaaacagatgcaattcccggacgtctaaaccaaaccactttcaccgctacacgaccgggggtatactacggtcaatgctctgaaatctgtggagcaaaccacagtttcatgcccatcgtcctagaattaattcccctaaaaatctttgaaatagggcccgtatttaccctatagcaccccctctaccccctctagagcccactgtaaagctaacttagcattaaccttttaagttaaagattaagagaaccaacacctctttacagtgaaatgccccaactaaatactaccgtatggcccaccataattacccccatactccttacactattcctcatcacccaactaaaaatattaaacacaaactaccacctacctccctcaccaaagcccataaaaataaaaaattataacaaaccctgagaaccaaaatgaacgaaaatctgttcgcttcattcattgcccccacaatcctaggcctacccgccgcagtactgatcattctatttccccctctattgatccccacctccaaatatctcatcaacaaccgactaatcaccacccaacaatgactaatcaaactaacctcaaaacaaatgataaccatacacaacactaaaggacgaacctgatctcttatactagtatccttaatcatttttattgccacaactaacctcctcggactcctgcctcactcatttacaccaaccacccaactatctataaacctagccatggccatccccttatgagcgggcgcagtgattataggctttcgctctaagattaaaaatgccctagcccacttcttaccacaaggcacacctacaccccttatccccatactagttattatcgaaaccatcagcctactcattcaaccaatagccctggccgtacgcctaaccgctaaca

SEQ ID NO: 6 - DNA, 2098 bp, Artificial Sequence
  nucleotide sequence of pMVA
gactcttcgcgatgtacgggccagatatacgccccattattcctagaaccaggcgacctgcgactccttgacgttgacaatcgagtagtactcccgattgaagcccccattcgtataataattacatcacaagacgtcttgcactcatgagccttctactgggcggttttatggacagcaagcgaaccggaattgccagctggggcgccctctggtaaggttgggaagccctgcaaagtaaactggatggctttctcgccgccaaggatctgatggcgcaggggatcaagctctgatcaagagacaggatgaggatcgtttcgcatgattgaacaagatggattgcacgcaggttctccggccgcttgggtggagaggctattcggctatgactgggcacaacagacaatcggctgctctgatgccgccgtgttccggctgtcagcgcaggggcgcccggttctttttgtcaagaccgacctgtccggtgccctgaatgaactgcaagacgaggcagcgcggctatcgtggctggccacgacgggcgttccttgcgcagctgtgctcgacgttgtcactgaagcgggaagggactggctgctattgggcgaagtgccggggcaggatctcctgtcatctcaccttgctcctgccgagaaagtatccatcatggctgatgcaatgcggcggctgcatacgcttgatccggctacctgcccattcgaccaccaagcgaaacatcgcatcgagcgagcacgtactcggatggaagccggtcttgtcgatcaggatgatctggacgaagagcatcaggggctcgcgccagccgaactgttcgccaggctcaaggcgagcatgcccgacggcgaggatctcgtcgtgacccatggcgatgcctgcttgccgaatatcatggtggaaaatggccgcttttctggattcatcgactgtggccggctgggtgtggcggaccgctatcaggacatagcgttggctacccgtgatattgctgaagagcttggcggcgaatgggctgaccgcttcctcgtgctttacggtatcgccgctcccgattcgcagcgcatcgccttctatcgccttcttgacgagttcttctgaattattaacgcttacaatttcctgatgcggtattttctccttacgcatctgtgcggtatttcacaccgcatacaggtggcacttttcggggaaatgtgcgcggaacccctatttgtttatttttctaaatacattcaaatatgtatccgctcatgagacaataaccctgataaatgcttcaataatagcacgtgctaaaacttcatttttaatttaaaaggatctaggtgaagatcctttttgataatctcatgaccaaaatcccttaacgtgagttttcgttccactgagcgtcagaccccgtagaaaagatcaaaggatcttcttgagatcctttttttctgcgcgtaatctgctgcttgcaaacaaaaaaaccaccgctaccagcggtggtttgtttgccggatcaagagctaccaactctttttccgaaggtaactggcttcagcagagcgcagataccaaatactgtccttctagtgtagccgtagttaggccaccacttcaagaactctgtagcaccgcctacatacctcgctctgctaatcctgttaccagtggctgctgccagtggcgataagtcgtgtcttaccgggttggactcaagacgatagttaccggataaggcgcagcggtcgggctgaacggggggttcgtgcacacagcccagcttggagcgaacgacctacaccgaactgagatacctacagcgtgagctatgagaaagcgccacgcttcccgaagggagaaaggcggacaggtatccggtaagcggcagggtcggaacaggagagcgcacgagggagcttccagggggaaacgcctggtatctttatagtcctgtcgggtttcgccacctctgacttgagcgtcgatttttgtgatgctcgtcaggggggcggagcctatggaaaaacgccagcaacgcggcctttttacggttcctgggcttttgctggccttttgctcacatgttctt

SEQ ID NO: 7 - DNA, 2578 bp, Artificial Sequence
  nucleotide sequence of pMVA
gactcttcgcgatgtacgggccagatatacgcctgaactatcctgcccgccatcatcctagtcctcatcgccctcccatccctacgcatcctttacataacagacgaggtcaacgatccctcccttaccatcaaatcaattggccaccaatggtactgaacctacgagtacaccgactacggcggactaatcttcaactcctacatacttcccccattattcctagaaccaggcgacctgcgactccttgacgttgacaatcgagtagtactcccgattgaagcccccattcgtataataattacatcacaagacgtcttgcactcatgagctgtccccacattaggcttaaaaacagatgcaattcccggacgtctaaaccaaaccactttcaccgctacacgaccgggggtatactacggtcaatgctctgaaatctgtggagcaaaccacagtttcatgcccatcgtcctagaattaattcccctaaaaatctttgaaatagggcccgtatttaccctatagcaccccctctaccccctctagagcccactgtaaagctaacttagcattaaccttttaagttaaagattaagagaaccaacacctctttacagtgaaatgccccaactcttctactgggcggttttatggacagcaagcgaaccggaattgccagctggggcgccctctggtaaggttgggaagccctgcaaagtaaactggatggctttctcgccgccaaggatctgatggcgcaggggatcaagctctgatcaagagacaggatgaggatcgtttcgcatgattgaacaagatggattgcacgcaggttctccggccgcttgggtggagaggctattcggctatgactgggcacaacagacaatcggctgctctgatgccgccgtgttccggctgtcagcgcaggggcgcccggttctttttgtcaagaccgacctgtccggtgccctgaatgaactgcaagacgaggcagcgcggctatcgtggctggccacgacgggcgttccttgcgcagctgtgctcgacgttgtcactgaagcgggaagggactggctgctattgggcgaagtgccggggcaggatctcctgtcatctcaccttgctcctgccgagaaagtatccatcatggctgatgcaatgcggcggctgcatacgcttgatccggctacctgcccattcgaccaccaagcgaaacatcgcatcgagcgagcacgtactcggatggaagccggtcttgtcgatcaggatgatctggacgaagagcatcaggggctcgcgccagccgaactgttcgccaggctcaaggcgagcatgcccgacggcgaggatctcgtcgtgacccatggcgatgcctgcttgccgaatatcatggtggaaaatggccgcttttctggattcatcgactgtggccggctgggtgtggcggaccgctatcaggacatagcgttggctacccgtgatattgctgaagagcttggcggcgaatgggctgaccgcttcctcgtgctttacggtatcgccgctcccgattcgcagcgcatcgccttctatcgccttcttgacgagttcttctgaattattaacgcttacaatttcctgatgcggtattttctccttacgcatctgtgcggtatttcacaccgcatacaggtggcacttttcggggaaatgtgcgcggaacccctatttgtttatttttctaaatacattcaaatatgtatccgctcatgagacaataaccctgataaatgcttcaataatagcacgtgctaaaacttcatttttaatttaaaaggatctaggtgaagatcctttttgataatctcatgaccaaaatcccttaacgtgagttttcgttccactgagcgtcagaccccgtagaaaagatcaaaggatcttcttgagatcctttttttctgcgcgtaatctgctgcttgcaaacaaaaaaaccaccgctaccagcggtggtttgtttgccggatcaagagctaccaactctttttccgaaggtaactggcttcagcagagcgcagataccaaatactgtccttctagtgtagccgtagttaggccaccacttcaagaactctgtagcaccgcctacatacctcgctctgctaatcctgttaccagtggctgctgccagtggcgataagtcgtgtcttaccgggttggactcaagacgatagttaccggataaggcgcagcggtcgggctgaacggggggttcgtgcacacagcccagcttggagcgaacgacctacaccgaactgagatacctacagcgtgagctatgagaaagcgccacgcttcccgaagggagaaaggcggacaggtatccggtaagcggcagggtcggaacaggagagcgcacgagggagcttccagggggaaacgcctggtatctttatagtcctgtcgggtttcgccacctctgacttgagcgtcgatttttgtgatgctcgtcaggggggcggagcctatggaaaaacgccagcaacgcggcctttttacggttcctgggcttttgctggccttttgctcacatgttctt

SEQ ID NO: 8 - DNA, 3978 bp, Artificial Sequence
  nucleotide sequence of pMVA
gactcttcgcgatgtacgggccagatatacgctacgttgtagctcacttccactatgtcctatcaataggagctgtatttgccatcataggaggcttcattcactgatttcccctattctcaggctacaccctagaccaaacctacgccaaaatccatttcactatcatattcatcggcgtaaatctaactttcttcccacaacactttctcggcctatccggaatgccccgacgttactcggactaccccgatgcatacaccacatgaaacatcctatcatctgtaggctcattcatttctctaacagcagtaatattaataattttcatgatttgagaagccttcgcttcgaagcgaaaagtcctaatagtagaagaaccctccataaacctggagtgactatatggatgccccccaccctaccacacattcgaagaacccgtatacataaaatctagacaaaaaaggaaggaatcgaaccccccaaagctggtttcaagccaaccccatggcctccatgactttttcaaaaaggtattagaaaaaccatttcataactttgtcaaagttaaattataggctaaatcctatatatcttaatggcacatgcagcgcaagtaggtctacaagacgctacttcccctatcatagaagagcttatcacctttcatgatcacgccctcataatcattttccttatctgcttcctagtcctgtatgcccttttcctaacactcacaacaaaactaactaatactaacatctcagacgctcaggaaatagaaaccgtctgaactatcctgcccgccatcatcctagtcctcatcgccctcccatccctacgcatcctttacataacagacgaggtcaacgatccctcccttaccatcaaatcaattggccaccaatggtactgaacctacgagtacaccgactacggcggactaatcttcaactcctacatacttcccccattattcctagaaccaggcgacctgcgactccttgacgttgacaatcgagtagtactcccgattgaagcccccattcgtataataattacatcacaagacgtcttgcactcatgagctgtccccacattaggcttaaaaacagatgcaattcccggacgtctaaaccaaaccactttcaccgctacacgaccgggggtatactacggtcaatgctctgaaatctgtggagcaaaccacagtttcatgcccatcgtcctagaattaattcccctaaaaatctttgaaatagggcccgtatttaccctatagcaccccctctaccccctctagagcccactgtaaagctaacttagcattaaccttttaagttaaagattaagagaaccaacacctctttacagtgaaatgccccaactaaatactaccgtatggcccaccataattacccccatactccttacactattcctcatcacccaactaaaaatattaaacacaaactaccacctacctccctcaccaaagcccataaaaataaaaaattataacaaaccctgagaaccaaaatgaacgaaaatctgttcgcttcattcattgcccccacaatcctaggcctacccgccgcagtactgatcattctatttccccctctattgatccccacctccaaatatctcatcaacaaccgactaatcaccacccaacaatgactaatcaaactaacctcaaaacaaatgataaccatacacaacactaaaggacgaacctgatctcttatactagtatccttaatcatttttattgccacaactaacctcctcggactcctgcctcactcatttacaccaaccacccaactatctataaacctagccatggccatccccttatgagcgggcgcagtgattataggctttcgctctaagattaaaaatgccctagcccacttcttaccacaaggcacacctacaccccttatccccatactagttattatcgaaaccatcagcctactcattcaaccaatagccctggccgtacgcctaaccgctaacacttctactgggcggttttatggacagcaagcgaaccggaattgccagctggggcgccctctggtaaggttgggaagccctgcaaagtaaactggatggctttctcgccgccaaggatctgatggcgcaggggatcaagctctgatcaagagacaggatgaggatcgtttcgcatgattgaacaagatggattgcacgcaggttctccggccgcttgggtggagaggctattcggctatgactgggcacaacagacaatcggctgctctgatgccgccgtgttccggctgtcagcgcaggggcgcccggttctttttgtcaagaccgacctgtccggtgccctgaatgaactgcaagacgaggcagcgcggctatcgtggctggccacgacgggcgttccttgcgcagctgtgctcgacgttgtcactgaagcgggaagggactggctgctattgggcgaagtgccggggcaggatctcctgtcatctcaccttgctcctgccgagaaagtatccatcatggctgatgcaatgcggcggctgcatacgcttgatccggctacctgcccattcgaccaccaagcgaaacatcgcatcgagcgagcacgtactcggatggaagccggtcttgtcgatcaggatgatctggacgaagagcatcaggggctcgcgccagccgaactgttcgccaggctcaaggcgagcatgcccgacggcgaggatctcgtcgtgacccatggcgatgcctgcttgccgaatatcatggtggaaaatggccgcttttctggattcatcgactgtggccggctgggtgtggcggaccgctatcaggacatagcgttggctacccgtgatattgctgaagagcttggcggcgaatgggctgaccgcttcctcgtgctttacggtatcgccgctcccgattcgcagcgcatcgccttctatcgccttcttgacgagttcttctgaattattaacgcttacaatttcctgatgcggtattttctccttacgcatctgtgcggtatttcacaccgcatacaggtggcacttttcggggaaatgtgcgcggaacccctatttgtttatttttctaaatacattcaaatatgtatccgctcatgagacaataaccctgataaatgcttcaataatagcacgtgctaaaacttcatttttaatttaaaaggatctaggtgaagatcctttttgataatctcatgaccaaaatcccttaacgtgagttttcgttccactgagcgtcagaccccgtagaaaagatcaaaggatcttcttgagatcctttttttctgcgcgtaatctgctgcttgcaaacaaaaaaaccaccgctaccagcggtggtttgtttgccggatcaagagctaccaactctttttccgaaggtaactggcttcagcagagcgcagataccaaatactgtccttctagtgtagccgtagttaggccaccacttcaagaactctgtagcaccgcctacatacctcgctctgctaatcctgttaccagtggctgctgccagtggcgataagtcgtgtcttaccgggttggactcaagacgatagttaccggataaggcgcagcggtcgggctgaacggggggttcgtgcacacagcccagcttggagcgaacgacctacaccgaactgagatacctacagcgtgagctatgagaaagcgccacgcttcccgaagggagaaaggcggacaggtatccggtaagcggcagggtcggaacaggagagcgcacgagggagcttccagggggaaacgcctggtatctttatagtcctgtcgggtttcgccacctctgacttgagcgtcgatttttgtgatgctcgtcaggggggcggagcctatggaaaaacgccagcaacgcggcctttttacggttcctgggcttttgctggccttttgctcacatgttctt

SEQ ID NO: 9 - DNA, 2097 bp, Artificial Sequence
  nucleotide sequence of pMVA
gctgcttcgcgatgtacgggccagatatacgccccattattcctagaaccaggcgacctgcgactccttgacgttgacaatcgagtagtactcccgattgaagcccccattcgtataataattacatcacaagacgtcttgcactcatgagccttctactgggcggttttatggacagcaagcgaaccggaattgccagctggggcgccctctggtaaggttgggaagccctgcaaagtaaactggatggctttcttgccgccaaggatctgatggcgcaggggatcaagctctgatcaagagacaggatgaggatcgtttcgcatgattgaacaagatggattgcacgcaggttctccggccgcttgggtggagaggctattcggctatgactgggcacaacagacaatcggctgctctgatgccgccgtgttccggctgtcagcgcaggggcgcccggttctttttgtcaagaccgacctgtccggtgccctgaatgaactgcaagacgaggcagcgcggctatcgtggctggccacgacgggcgttccttgcgcagctgtgctcgacgttgtcactgaagcgggaagggactggctgctattgggcgaagtgccggggcaggatctcctgtcatctcaccttgctcctgccgagaaagtatccatcatggctgatgcaatgcggcggctgcatacgcttgatccggctacctgcccattcgaccaccaagcgaaacatcgcatcgagcgagcacgtactcggatggaagccggtcttgtcgatcaggatgatctggacgaagagcatcaggggctcgcgccagccgaactgttcgccaggctcaaggcgagcatgcccgacggcgaggatctcgtcgtgacccatggcgatgcctgcttgccgaatatcatggtggaaaatggccgcttttctggattcatcgactgtggccggctgggtgtggcggaccgctatcaggacatagcgttggctacccgtgatattgctgaagagcttggcggcgaatgggctgaccgcttcctcgtgctttacggtatcgccgctcccgattcgcagcgcatcgccttctatcgccttcttgacgagttcttctgaattattaacgcttacaatttcctgatgcggtattttctccttacgcatctgtgcggtatttcacaccgcatcaggtggcacttttcggggaaatgtgcgcggaacccctatttgtttatttttctaaatacattcaaatatgtatccgctcatgagacaataaccctgataaatgcttcaataatagcacgtgctaaaacttcatttttaatttaaaaggatctaggtgaagatcctttttgataatctcatgaccaaaatcccttaacgtgagttttcgttccactgagcgtcagaccccgtagaaaagatcaaaggatcttcttgagatcctttttttctgcgcgtaatctgctgcttgcaaacaaaaaaaccaccgctaccagcggtggtttgtttgccggatcaagagctaccaactctttttccgaaggtaactggcttcagcagagcgcagataccaaatactgttcttctagtgtagccgtagttaggccaccacttcaagaactctgtagcaccgcctacatacctcgctctgctaatcctgttaccagtggctgctgccagtggcgataagtcgtgtcttaccgggttggactcaagacgatagttaccggataaggcgcagcggtcgggctgaacggggggttcgtgcacacagcccagcttggagcgaacgacctacaccgaactgagatacctacagcgtgagctatgagaaagcgccacgcttcccgaagggagaaaggcggacaggtatccggtaagcggcagggtcggaacaggagagcgcacgagggagcttccagggggaaacgcctggtatctttatagtcctgtcgggtttcgccacctctgacttgagcgtcgatttttgtgatgctcgtcaggggggcggagcctatggaaaaacgccagcaacgcggcctttttacggttcctggccttttgctggccttttgctcacatgttctt

SEQ ID NO: 10 - DNA, 2577 bp, Artificial Sequence
  nucleotide sequence of pMVA
gctgcttcgcgatgtacgggccagatatacgcctgaactatcctgcccgccatcatcctagtcctcatcgccctcccatccctacgcatcctttacataacagacgaggtcaacgatccctcccttaccatcaaatcaattggccaccaatggtactgaacctacgagtacaccgactacggcggactaatcttcaactcctacatacttcccccattattcctagaaccaggcgacctgcgactccttgacgttgacaatcgagtagtactcccgattgaagcccccattcgtataataattacatcacaagacgtcttgcactcatgagctgtccccacattaggcttaaaaacagatgcaattcccggacgtctaaaccaaaccactttcaccgctacacgaccgggggtatactacggtcaatgctctgaaatctgtggagcaaaccacagtttcatgcccatcgtcctagaattaattcccctaaaaatctttgaaatagggcccgtatttaccctatagcaccccctctaccccctctagagcccactgtaaagctaacttagcattaaccttttaagttaaagattaagagaaccaacacctctttacagtgaaatgccccaactcttctactgggcggttttatggacagcaagcgaaccggaattgccagctggggcgccctctggtaaggttgggaagccctgcaaagtaaactggatggctttcttgccgccaaggatctgatggcgcaggggatcaagctctgatcaagagacaggatgaggatcgtttcgcatgattgaacaagatggattgcacgcaggttctccggccgcttgggtggagaggctattcggctatgactgggcacaacagacaatcggctgctctgatgccgccgtgttccggctgtcagcgcaggggcgcccggttctttttgtcaagaccgacctgtccggtgccctgaatgaactgcaagacgaggcagcgcggctatcgtggctggccacgacgggcgttccttgcgcagctgtgctcgacgttgtcactgaagcgggaagggactggctgctattgggcgaagtgccggggcaggatctcctgtcatctcaccttgctcctgccgagaaagtatccatcatggctgatgcaatgcggcggctgcatacgcttgatccggctacctgcccattcgaccaccaagcgaaacatcgcatcgagcgagcacgtactcggatggaagccggtcttgtcgatcaggatgatctggacgaagagcatcaggggctcgcgccagccgaactgttcgccaggctcaaggcgagcatgcccgacggcgaggatctcgtcgtgacccatggcgatgcctgcttgccgaatatcatggtggaaaatggccgcttttctggattcatcgactgtggccggctgggtgtggcggaccgctatcaggacatagcgttggctacccgtgatattgctgaagagcttggcggcgaatgggctgaccgcttcctcgtgctttacggtatcgccgctcccgattcgcagcgcatcgccttctatcgccttcttgacgagttcttctgaattattaacgcttacaatttcctgatgcggtattttctccttacgcatctgtgcggtatttcacaccgcatcaggtggcacttttcggggaaatgtgcgcggaacccctatttgtttatttttctaaatacattcaaatatgtatccgctcatgagacaataaccctgataaatgcttcaataatagcacgtgctaaaacttcatttttaatttaaaaggatctaggtgaagatcctttttgataatctcatgaccaaaatcccttaacgtgagttttcgttccactgagcgtcagaccccgtagaaaagatcaaaggatcttcttgagatcctttttttctgcgcgtaatctgctgcttgcaaacaaaaaaaccaccgctaccagcggtggtttgtttgccggatcaagagctaccaactctttttccgaaggtaactggcttcagcagagcgcagataccaaatactgttcttctagtgtagccgtagttaggccaccacttcaagaactctgtagcaccgcctacatacctcgctctgctaatcctgttaccagtggctgctgccagtggcgataagtcgtgtcttaccgggttggactcaagacgatagttaccggataaggcgcagcggtcgggctgaacggggggttcgtgcacacagcccagcttggagcgaacgacctacaccgaactgagatacctacagcgtgagctatgagaaagcgccacgcttcccgaagggagaaaggcggacaggtatccggtaagcggcagggtcggaacaggagagcgcacgagggagcttccagggggaaacgcctggtatctttatagtcctgtcgggtttcgccacctctgacttgagcgtcgatttttgtgatgctcgtcaggggggcggagcctatggaaaaacgccagcaacgcggcctttttacggttcctggccttttgctggccttttgctcacatgttctt

SEQ ID NO: 11 - DNA, 3977 bp, Artificial Sequence
  nucleotide sequence of pMVA
gctgcttcgcgatgtacgggccagatatacgctacgttgtagctcacttccactatgtcctatcaataggagctgtatttgccatcataggaggcttcattcactgatttcccctattctcaggctacaccctagaccaaacctacgccaaaatccatttcactatcatattcatcggcgtaaatctaactttcttcccacaacactttctcggcctatccggaatgccccgacgttactcggactaccccgatgcatacaccacatgaaacatcctatcatctgtaggctcattcatttctctaacagcagtaatattaataattttcatgatttgagaagccttcgcttcgaagcgaaaagtcctaatagtagaagaaccctccataaacctggagtgactatatggatgccccccaccctaccacacattcgaagaacccgtatacataaaatctagacaaaaaaggaaggaatcgaaccccccaaagctggtttcaagccaaccccatggcctccatgactttttcaaaaaggtattagaaaaaccatttcataactttgtcaaagttaaattataggctaaatcctatatatcttaatggcacatgcagcgcaagtaggtctacaagacgctacttcccctatcatagaagagcttatcacctttcatgatcacgccctcataatcattttccttatctgcttcctagtcctgtatgcccttttcctaacactcacaacaaaactaactaatactaacatctcagacgctcaggaaatagaaaccgtctgaactatcctgcccgccatcatcctagtcctcatcgccctcccatccctacgcatcctttacataacagacgaggtcaacgatccctcccttaccatcaaatcaattggccaccaatggtactgaacctacgagtacaccgactacggcggactaatcttcaactcctacatacttcccccattattcctagaaccaggcgacctgcgactccttgacgttgacaatcgagtagtactcccgattgaagcccccattcgtataataattacatcacaagacgtcttgcactcatgagctgtccccacattaggcttaaaaacagatgcaattcccggacgtctaaaccaaaccactttcaccgctacacgaccgggggtatactacggtcaatgctctgaaatctgtggagcaaaccacagtttcatgcccatcgtcctagaattaattcccctaaaaatctttgaaatagggcccgtatttaccctatagcaccccctctaccccctctagagcccactgtaaagctaacttagcattaaccttttaagttaaagattaagagaaccaacacctctttacagtgaaatgccccaactaaatactaccgtatggcccaccataattacccccatactccttacactattcctcatcacccaactaaaaatattaaacacaaactaccacctacctccctcaccaaagcccataaaaataaaaaattataacaaaccctgagaaccaaaatgaacgaaaatctgttcgcttcattcattgcccccacaatcctaggcctacccgccgcagtactgatcattctatttccccctctattgatccccacctccaaatatctcatcaacaaccgactaatcaccacccaacaatgactaatcaaactaacctcaaaacaaatgataaccatacacaacactaaaggacgaacctgatctcttatactagtatccttaatcatttttattgccacaactaacctcctcggactcctgcctcactcatttacaccaaccacccaactatctataaacctagccatggccatccccttatgagcgggcgcagtgattataggctttcgctctaagattaaaaatgccctagcccacttcttaccacaaggcacacctacaccccttatccccatactagttattatcgaaaccatcagcctactcattcaaccaatagccctggccgtacgcctaaccgctaacacttctactgggcggttttatggacagcaagcgaaccggaattgccagctggggcgccctctggtaaggttgggaagccctgcaaagtaaactggatggctttcttgccgccaaggatctgatggcgcaggggatcaagctctgatcaagagacaggatgaggatcgtttcgcatgattgaacaagatggattgcacgcaggttctccggccgcttgggtggagaggctattcggctatgactgggcacaacagacaatcggctgctctgatgccgccgtgttccggctgtcagcgcaggggcgcccggttctttttgtcaagaccgacctgtccggtgccctgaatgaactgcaagacgaggcagcgcggctatcgtggctggccacgacgggcgttccttgcgcagctgtgctcgacgttgtcactgaagcgggaagggactggctgctattgggcgaagtgccggggcaggatctcctgtcatctcaccttgctcctgccgagaaagtatccatcatggctgatgcaatgcggcggctgcatacgcttgatccggctacctgcccattcgaccaccaagcgaaacatcgcatcgagcgagcacgtactcggatggaagccggtcttgtcgatcaggatgatctggacgaagagcatcaggggctcgcgccagccgaactgttcgccaggctcaaggcgagcatgcccgacggcgaggatctcgtcgtgacccatggcgatgcctgcttgccgaatatcatggtggaaaatggccgcttttctggattcatcgactgtggccggctgggtgtggcggaccgctatcaggacatagcgttggctacccgtgatattgctgaagagcttggcggcgaatgggctgaccgcttcctcgtgctttacggtatcgccgctcccgattcgcagcgcatcgccttctatcgccttcttgacgagttcttctgaattattaacgcttacaatttcctgatgcggtattttctccttacgcatctgtgcggtatttcacaccgcatcaggtggcacttttcggggaaatgtgcgcggaacccctatttgtttatttttctaaatacattcaaatatgtatccgctcatgagacaataaccctgataaatgcttcaataatagcacgtgctaaaacttcatttttaatttaaaaggatctaggtgaagatcctttttgataatctcatgaccaaaatcccttaacgtgagttttcgttccactgagcgtcagaccccgtagaaaagatcaaaggatcttcttgagatcctttttttctgcgcgtaatctgctgcttgcaaacaaaaaaaccaccgctaccagcggtggtttgtttgccggatcaagagctaccaactctttttccgaaggtaactggcttcagcagagcgcagataccaaatactgttcttctagtgtagccgtagttaggccaccacttcaagaactctgtagcaccgcctacatacctcgctctgctaatcctgttaccagtggctgctgccagtggcgataagtcgtgtcttaccgggttggactcaagacgatagttaccggataaggcgcagcggtcgggctgaacggggggttcgtgcacacagcccagcttggagcgaacgacctacaccgaactgagatacctacagcgtgagctatgagaaagcgccacgcttcccgaagggagaaaggcggacaggtatccggtaagcggcagggtcggaacaggagagcgcacgagggagcttccagggggaaacgcctggtatctttatagtcctgtcgggtttcgccacctctgacttgagcgtcgatttttgtgatgctcgtcaggggggcggagcctatggaaaaacgccagcaacgcggcctttttacggttcctggccttttgctggccttttgctcacatgttctt